European Patent Specification EP 4 065 154 B1, published May 20, 2026. Title: UK 114 SALMON PROTEINS FOR USE IN THE TREATMENT, DIAGNOSIS AND PREVENTION OF MALIGNANT TUMOURS. Applicant: Bartorelli Cusani, Alberto. The sequence listing filed with the application follows.

SEQUENCE LISTING (6 sequences)

SEQ ID NO: 1 - protein, 139 aa, Salmo salar
GSHMSSIIRKIINTSKAPAAIGPYSQAVVVDRTMYVSGQLGMDPASGQLVEGGVQAQTKQALVNMGEILKEAGCGYDSVVKTTVLLADMNDFASVNDVYKTFFSSSFPARAAYQVAALPRGGLVEIEAVAVLGPLTEVS

SEQ ID NO: 2 - protein, 138 aa, Salmo salar
GSHMAAVQKLFPYTPRAPIRQGIYSQAVVVDRTMYISGQLGLDVASGKLVEGGVQAQARQALVNMGEILKAAGCGYDNVVKTTVLLADMNDFVNVNDVYKTFFSKNFPARAAYQVVALPRGGLVEIEAVAVLGPISES

SEQ ID NO: 3 - DNA, 471 bp, Salmo salar
atgggcagcagccatcatcatcatcatcacagcagcggcctggtgccgcgcggcagccatatgtcttcgatcatcaggaagataattaacaccagtaaagcgccagcagctatcgggccgtacagccaggcggtggtggtggacaggaccatgtacgtgtcaggccagctggggatggaccctgcctctggtcagctggtggaaggaggagtccaggctcagaccaaacaggctctggtgaacatgggggagatcctgaaagaagcagggtgtggatatgacagtgtcgtgaaaactacggttcttttggctgacatgaatgacttcgccagtgtaaatgacgtctataaaacatttttcagcagtagcttcccagcgagggctgcctaccaggtcgctgctctgcccaggggtgggcttgtagagattgaagctgtggctgttctaggccctctgactgaggtctcttga

SEQ ID NO: 4 - DNA, 468 bp, Salmo salar
atgggcagcagccatcatcatcatcatcacagcagcggcctggtgccgcgcggcagccatatggctgctgttcagaaactctttccttatactcctagagcacctataaggcaggggatttacagccaggcggtggtggtggatcggacgatgtacatctccggccagctggggctggacgtggcctcagggaagctggtggagggaggggtacaggctcaggccagacaggctctggtcaatatgggagagatcctgaaagcagctggatgtggttatgacaatgtcgtcaagacaaccgtgctgttggcagacatgaatgactttgtcaatgtcaacgatgtttataagacatttttcagcaaaaacttccctgccagagctgcctaccaggttgttgccctccccagaggtggcctggtggagatcgaggctgtggctgttctgggacccatctctgagtcctga

SEQ ID NO: 5 - protein, 156 aa, Salmo salar
MGSSHHHHHHSSGLVPRGSHMSSIIRKIINTSKAPAAIGPYSQAVVVDRTMYVSGQLGMDPASGQLVEGGVQAQTKQALVNMGEILKEAGCGYDSVVKTTVLLADMNDFASVNDVYKTFFSSSFPARAAYQVAALPRGGLVEIEAVAVLGPLTEVS

SEQ ID NO: 6 - protein, 155 aa, Salmo salar
MGSSHHHHHHSSGLVPRGSHMAAVQKLFPYTPRAPIRQGIYSQAVVVDRTMYISGQLGLDVASGKLVEGGVQAQARQALVNMGEILKAAGCGYDNVVKTTVLLADMNDFVNVNDVYKTFFSKNFPARAAYQVVALPRGGLVEIEAVAVLGPISES